European Patent Application EP 4 534 668 A1, published April 9, 2025. Title: がんを処置するための組成物. Applicant: Kyoto University. The sequence listing filed with the application follows.

SEQUENCE LISTING (41 sequences)

SEQ ID NO: 1 - protein, 618 aa, Homo sapiens
MGVGRQQRGPFQGVRVKNSVKELLLHIRSHKQKASGQAVDDFKTQGVNIEQFRELKNTVSYSGKRKGPDSLSDGPACKRPALLHSQFLTPPQTPTPGESMEDVHLNEPKQESSADLLQNIINIKNECSPVSLNTVQVSWLNPVVVPQSSPAEQCQDFHGGQVFSPPQKCQPFQVRGSQQMIDQASLYQYSPQNQHVEQQPHYTHKPTLEYSPFPIPPQSPAYEPNLFDGPESQFCPNQSLVSLLGDQRESENIANPMQTSSSVQQQNDAHLHSFSMMPSSACEAMVGHEMASDSSNTSLPFSNMGNPMNTTQLGKSLFQWQVEQEESKLANISQDQFLSKDADGDTFLHIAVAQGRRALSYVLARKMNALHMLDIKEHNGQSAFQVAVAANQHLIVQDLVNIGAQVNTTDCWGRTPLHVCAEKGHSQVLQAIQKGAVGSNQFVDLEATNYDGLTPLHCAVIAHNAVVHELQRNQQPHSPEVQELLLKNKSLVDTIKCLIQMGAAVEAKDRKSGRTALHLAAEEANLELIRLFLELPSCLSFVNAKAYNGNTALHVAASLQYRLTQLDAVRLLMRKGADPSTRNLENEQPVHLVPDGPVGEQIRRILKGKSIQQRAPPY

SEQ ID NO: 2 - protein, 728 aa, Mus musculus
MIVDKLLDDSRGGEGLLDAAGDCGLMTSPLNLAYFYGASPPSAPGAGDTGYLSAVPSAPGSPGSDSSDFSSTSSVSSCGAVESRPRGGARAERPQVEPHMGVGRQQRGPFQGVRVKNSVKELLLHIRSNKQKASGQPVDEFKTQSVNIEQLTDLKSAVSAVGKRKGPDPLSDGPVCKRPALLPSHFVTSPQTPTPGESMEDVRHSESKLDSSAALLQNIINIKNECNPVSLNTVQVSWMSPTVPQNSPRDQCQDFHGGQAFSPPQKYQPFQVSGSPQMMDQASMYQYSPQTQNMQQPPPLPPQQQHQQNYPHNSPLQFSPYSRMSQSPKYDSNLFDTHEPQFCTGQSFVSLLTGPGEPESLAVPVPAPTSIPPQTETQLQTFSLMPSNACEAVVGVHDVGSHSLGTSLSLQNIMGSPMNTTQLGKSFFQWQVEQEESKLANIPQDQFLARDGDGDTFLHIAVAQGRRALSYVLARKMNALHMLDIKEHNGQSAFQVAVAANQHLIVQDLVNLGAQVNTTDCWGRTPLHVCAEKGHSQVLQAIQKGAVRSNQFVDLEATNYDGLTPLHCAVVAHNAVVHELQRNRQSHSPEVQDLLLRNKSLVDTIKCLIQMGAAVEAKDRKSGRTALHLAAEEANLELIRLFLELPSCLSFVNAKAYNGNTALHVAASLQYRVTQLDAVRLLMRKGADPSTRNLENEQPVHLVPDGPVGEQIRRILKGKSIQQRAPPY

SEQ ID NO: 3 - RNA, 3790 nt, Homo sapiens
  source 1..3790: mol_type = mRNA
ctcctcttgccacgaggtcagacggcgagttcttagagaaaaaggctgcttagctgctgcttatcatgtaacctcaaaaggaaactgatcgtctttctcatgctgtcacgtacttgggttattatcgctgattacagctggaaacaattgatttgctcttacgtatttgtgtgacttgactcttcaaacacaaaggttaacaggaagatctcgagggccctggctgaacttcaccttttggctttcttggcctgatgctgaactctcgaggttgagccccatatgggggttggcaggcagcagagaggcccctttcaaggtgttcgggtaaagaactcagtgaaggaactcctgttgcacatccgaagtcataaacagaaggcttctggccaagctgtggatgattttaagacacaaggtgtgaacatagaacagttcagagaattgaagaacacagtatcatacagtgggaaaaggaaagggcccgattcgttgtctgatggacctgcttgcaaaaggccagctctgttgcattcccaatttttgacaccacctcaaacaccaacgcccggggagagcatggaagatgttcatctcaatgaacccaaacaggagagcagtgctgatctgcttcagaacattatcaacattaagaatgaatgcagccccgtttccctgaacacagttcaagttagctggctgaaccccgtggtggtccctcagagctcccccgcagagcagtgtcaggacttccatggagggcaggtcttttctccacctcagaaatgccaaccattccaagtcaggggctcccaacaaatgatagaccaggcttccctgtaccagtattctccacagaaccagcatgtagagcagcagccacactacacccacaaaccaactctggaatacagtccttttcccatacctccccagtcccccgcttatgaaccaaacctctttgatggtccagaatcacagttttgcccaaaccaaagcttagtttcccttcttggtgatcaaagggaatctgagaatattgctaatcccatgcagacttcctccagtgttcagcagcaaaatgatgctcacttgcacagcttcagcatgatgcccagcagcgcctgtgaggccatggtggggcacgagatggcctctgactcttcaaacacttcactgccattctcaaacatgggaaatccaatgaacaccacacagttagggaaatcactttttcagtggcaggtggagcaggaagaaagcaaattggcaaatatttcccaagaccagtttctttcaaaggatgcagatggtgacacgttccttcatattgctgttgcccaagggagaagggcactttcctatgttcttgcaagaaagatgaatgcacttcacatgctggatattaaagagcacaatggacagagtgcctttcaggtggcagtggctgccaatcagcatctcattgtgcaggatctggtgaacatcggggcacaggtgaacaccacagactgctggggaagaacacctctgcatgtgtgtgctgagaagggccactcccaggtgcttcaggcgattcagaagggagcagtgggaagtaatcagtttgtggatcttgaggcaactaactatgatggcctgactccccttcactgtgcagtcatagcccacaatgctgtggtccatgaactccagagaaatcaacagcctcattcacctgaagttcaggagcttttactgaagaataagagtctggttgataccattaagtgcctaattcaaatgggagcagcggtggaagcgaaggatcgcaaaagtggccgcacagccctgcatttggcagctgaagaagcaaatctggaactcattcgcctctttttggagctgcccagttgcctgtcttttgtgaatgcaaaggcttacaatggcaacactgccctccatgttgctgccagcttgcagtatcggttgacacaattagatgctgtccgcctgttgatgaggaagggagcagacccaagtactcggaacttggagaacgaacagccagtgcatttggttcccgatggccctgtgggagaacagatccgacgtatcctgaagggaaagtccattcagcagagagctccaccgtattagctccattagcttggagcctggctagcaacactcactgtcagttaggcagtcctgatgtatctgtacatagaccatttgccttatattggcaaatgtaagttgtttctatgaaacaaacatatttagttcactattatatagtgggttatattaaaagaaaagaagaaaaatatctaatttctcttggcagatttgcatatttcatacccaggtatctgggatctagacatctgaatttgatctcaatggtaacattgccttcaattaacagtagcttttgagtaggaaaggactttgatttgtggcacaaaacattattaatatagctattgacagtttcaaagcaggtaaattgtaaatgtttctttaagaaaaagcatgtgaaaggaaaaaggtaaatacagcattgaggcttcatttggccttagtccctgggagttactggcgttggacaggcttcagtcattggactagatgaaaggtgtccatggttagaatttgatctttgcaaactgtatataattgttatttttgtccttaaaaatattgtacatacttggttgttaacatggtcatatttgaaatgtataagtccataaaatagaaaagaacaagtgaattgttgctatttaaaaaaattttacaattcttactaaggagtttttattgtgtaatcactaagtctttgtagataaagcagatggggagttacggagttgttcctttactggctgaaagatatattcgaattgtaaagatgctttttctcatgcattgaaattatacattatttgtagggaattgcatgcttttttttttttttctcccgagacagggtcttgctctggcgcccaggctggagtacagtggcatgatcttggctcacttcagccttgacttgggctcaagtgatcctcctacctgagccttctgagtaactggaactacaggtgtgcactcctcgcctggctaattttttattttttgtacaggcaggatcttgccaccttgcccaggctggtcttgaactcctgagctcatgccatctgcctgccttagtctcccaaaatgctgggattacaggagtgagccaccatgcccggctggcagttgcatggaagagaacacctctttatggcttaccctctagaatttctaatttatgtgttctgttgaaatttttgtttttttacctttattgaaacaacaaaaagtcagtattgaaacatatcttcctgttttctgttgtcaaatgatgataatgtgccatgatgttttatatatatcattcagaaaaagttttattttttaataacattctattaacattattttgcttgccgctggcatgcctgaggaatgtatttggctttgattacacactaagtttttgtaataaatttgactcattaaaaaccttttttttttaaaaaaaaaaaaaaagaaaatctcattagtgaacttatctttgcagctgagtacttaaattctttttaaaaagataccctttggattgatcacattgtttgacccagtatgtcttgtagacacgttagttataatcaccttgtatctctaaatatggtgtgatatgaaccagtccattcacattggaaaaactgatggttttaaataaactaattcactaata

SEQ ID NO: 4 - RNA, 3625 nt, Mus musculus
  source 1..3625: mol_type = mRNA
acgtactagtcgctctgccgcagccaaccgcgtagccatccggtggcgcaggtgtctggggaccccgagcgcctagcctgggagcatgatcgtggacaagctgctggacgacagccgcggcggagaggggctgctggacgcggccggcgactgcggcctcatgaccagcccgctcaacctggcttacttctacggcgcctcgcctccttccgcccccggcgccggcgacaccggctacctgtccgccgtgccctccgcgcccggctcgcccggctccgactcctccgatttctcctccacttcctccgtgtcctcctgcggggccgtggagtcccgtcccagaggtggcgcccgcgccgagcgccctcaagttgagccccacatgggggttggcaggcagcagagaggcccctttcaaggtgttcgcgtgaagaactcggtgaaggagctcctgctacacatccgaagcaacaagcagaaggcttccggccagcccgtggatgagtttaagacacagagtgtgaacattgagcagctgacagacctgaagagtgcagtgtccgcagtggggaaaagaaagggacccgatcctctgtccgatggaccggtttgcaagaggccagctctgttgccttctcacttcgtgacatcaccgcaaacgcctacacctggggagagcatggaagatgttcgccacagcgaatccaagctggatagcagcgctgccctgcttcagaatattataaacatcaagaatgagtgcaacccagtttcactaaacactgttcaggttagctggatgagccccacggttccccagaactcgccaagagaccagtgccaggatttccatggaggccaggccttctctccacctcagaaataccaaccgttccaagtcagtggctctccacagatgatggaccaggcgtcaatgtaccagtattcgccacaaacacagaacatgcagcagccgccgccgctgccaccacagcagcaacatcaacagaattatccccacaactcacccctgcagttcagtccttactccagaatgtcccagtctcccaagtatgattccaacctctttgatactcacgagccacagttctgcacgggccaaagttttgtgtctttactgactggcccgggggaacccgagtctcttgctgttcccgttccggctcccaccagcattccaccccaaactgagactcagctgcagaccttcagcctgatgccaagcaatgcctgcgaggccgtcgtcggggtgcacgatgtgggctcgcactctttgggcacgtccctgtcactccagaacatcatgggaagcccgatgaataccacccagctggggaagtcattttttcagtggcaggtagagcaggaagaaagcaaattggcaaatattccccaggaccagttcctcgctagggacggagatggtgacacgtttctccatattgctgttgcccaagggaggcgagcgctctcgtatgtccttgcaagaaagatgaacgctcttcacatgctggacattaaggagcacaatggacagagtgcctttcaggtggcggtagctgccaatcagcacctcattgtgcaagatctggtaaaccttggtgcccaggtgaacaccacggattgctggggaaggacacctctgcatgtctgtgcggagaagggccactcccaggtgctccaggccatccagaagggagctgtgaggagcaatcagtttgtggatcttgaggcaacgaactatgatggcctgactcccctacattgcgcggtcgtggctcacaatgcggtggtgcacgaactgcagaggaatcggcagtctcattcgcccgaagtgcaggacctcttactaaggaataagagcctggtagacaccattaagtgtctgattcagatgggagccgcagtggaggcaaaggatcgtaagagtggccgcacagccctgcacttggcagcggaagaagcaaatctggaactcattcgcctctttttggagttgcccagttgcctgtctttcgtgaatgccaaggcttacaatggaaacaccgccctccatgttgctgccagcctgcagtatcgggtgacacagttggacgcagtccgcctgttgatgaggaagggagctgaccccagtactcggaacttggagaatgaacagcccgtgcatttggtccccgatggcccagtgggagaacagatccgacgtatcctgaaggggaagtccattcagcagcgagcaccaccatactaggtccactggcgtggagcctggttcagcgacactcactgtcagttaggcagtcctgatgtatctgtacatagaccatttgccctgtattggcaaatgtaagttgtttctatgaaacaaacccatttagttcactattatatagtggattatattaaaagaaaagaagacagatatctaattttcttggcagatttgcgtatttcatacccaggtatctgggatctatatatctgaatttgatcttgaatggtaaaattaccttcgataaccagtagctttcaggtagggaaaaaaaaaaagactcatgggaaaagacttgatctgtggcataaagccttgctcatgtagagattgccaggtccagattaggtgggcttgaaacatgaggtgaaaaatgaaagcatttgaaaggggacagaaatttggatgtgaggttgatgtgcactttgctgtcatcgatgcttctttggtcagatgcaggacctggtgtttaataatgctctctctctaggtgagggaggcctcttgataggatgtgatctttgaagctgtatataattctcatttttaccttttaaaatgttgtacatatttgatttgaaccacggacatttgaaatgtgtaagtcaatcaagtagaaaagagctagtgaattgttcaccactttcaaggttgtgcacccacaaagcaacttgtactgtgtaatcgtccagctagagtttttacagataaagcaaatggggaagtgggtcccaacgttgctgtggtagcaggcgggtttctcttgcattggaaacagacacgtttgtaggcatttgcgtattcttgaagagactgttttatgaatcacctcttagatttatgtaatttacctaagttgttgaagtttctgtttctccttaagagaaattacaaaaattcaacattgaagcatagtttcttgttttctgttgtcaaatagtaataatgtgctgtgatgtttatgcttattcataaagatgttttactttttagtgtaatgttagttcttttaacattattttgcttaaatttgataatgcccgacaagaatatattttgctttgatttatacactgattctttgtgacaaatatgacccattaaaaatgccttttaatagactaacttaccttttgtagctaggtactcatgttcttttttaaaagatgccctttggattggattggattgatcatgtttaactcagcgtattttatggatgaaagctaaatacagatatttggcatctctaaggtggaatgagcccactccacacactgataaaattcatgcatagttttaaatgaacattaataaactcatgttgtctta

SEQ ID NO: 5 - RNA, 44 nt, Homo sapiens
  source 1..44: mol_type = mRNA
ttgtttctatgaaacaaacatatttagttcactattatatagtg

SEQ ID NO: 6 - RNA, 44 nt, Mus musculus
  source 1..44: mol_type = mRNA
ttgtttctatgaaacaaacccatttagttcactattatatagtg

SEQ ID NO: 7 - RNA, 110 nt, Homo sapiens
  source 1..110: mol_type = mRNA
actgtcagttaggcagtcctgatgtatctgtacatagaccatttgccttatattggcaaatgtaagttgtttctatgaaacaaacatatttagttcactattatatagtg

SEQ ID NO: 8 - RNA, 110 nt, Mus musculus
  source 1..110: mol_type = mRNA
actgtcagttaggcagtcctgatgtatctgtacatagaccatttgccctgtattggcaaatgtaagttgtttctatgaaacaaacccatttagttcactattatatagtg

SEQ ID NO: 9 - RNA, 1651 nt, Homo sapiens
  source 1..1651: mol_type = mRNA
ctccattagcttggagcctggctagcaacactcactgtcagttaggcagtcctgatgtatctgtacatagaccatttgccttatattggcaaatgtaagttgtttctatgaaacaaacatatttagttcactattatatagtgggttatattaaaagaaaagaagaaaaatatctaatttctcttggcagatttgcatatttcatacccaggtatctgggatctagacatctgaatttgatctcaatggtaacattgccttcaattaacagtagcttttgagtaggaaaggactttgatttgtggcacaaaacattattaatatagctattgacagtttcaaagcaggtaaattgtaaatgtttctttaagaaaaagcatgtgaaaggaaaaaggtaaatacagcattgaggcttcatttggccttagtccctgggagttactggcgttggacaggcttcagtcattggactagatgaaaggtgtccatggttagaatttgatctttgcaaactgtatataattgttatttttgtccttaaaaatattgtacatacttggttgttaacatggtcatatttgaaatgtataagtccataaaatagaaaagaacaagtgaattgttgctatttaaaaaaattttacaattcttactaaggagtttttattgtgtaatcactaagtctttgtagataaagcagatggggagttacggagttgttcctttactggctgaaagatatattcgaattgtaaagatgctttttctcatgcattgaaattatacattatttgtagggaattgcatgcttttttttttttttctcccgagacagggtcttgctctggcgcccaggctggagtacagtggcatgatcttggctcacttcagccttgacttgggctcaagtgatcctcctacctgagccttctgagtaactggaactacaggtgtgcactcctcgcctggctaattttttattttttgtacaggcaggatcttgccaccttgcccaggctggtcttgaactcctgagctcatgccatctgcctgccttagtctcccaaaatgctgggattacaggagtgagccaccatgcccggctggcagttgcatggaagagaacacctctttatggcttaccctctagaatttctaatttatgtgttctgttgaaatttttgtttttttacctttattgaaacaacaaaaagtcagtattgaaacatatcttcctgttttctgttgtcaaatgatgataatgtgccatgatgttttatatatatcattcagaaaaagttttattttttaataacattctattaacattattttgcttgccgctggcatgcctgaggaatgtatttggctttgattacacactaagtttttgtaataaatttgactcattaaaaaccttttttttttaaaaaaaaaaaaaaagaaaatctcattagtgaacttatctttgcagctgagtacttaaattctttttaaaaagataccctttggattgatcacattgtttgacccagtatgtcttgtagacacgttagttataatcaccttgtatctctaaatatggtgtgatatgaaccagtccattcacattggaaaaactgatggttttaaataaactaattcactaata

SEQ ID NO: 10 - RNA, 1353 nt, Mus musculus
  source 1..1353: mol_type = mRNA
gtccactggcgtggagcctggttcagcgacactcactgtcagttaggcagtcctgatgtatctgtacatagaccatttgccctgtattggcaaatgtaagttgtttctatgaaacaaacccatttagttcactattatatagtggattatattaaaagaaaagaagacagatatctaattttcttggcagatttgcgtatttcatacccaggtatctgggatctatatatctgaatttgatcttgaatggtaaaattaccttcgataaccagtagctttcaggtagggaaaaaaaaaaagactcatgggaaaagacttgatctgtggcataaagccttgctcatgtagagattgccaggtccagattaggtgggcttgaaacatgaggtgaaaaatgaaagcatttgaaaggggacagaaatttggatgtgaggttgatgtgcactttgctgtcatcgatgcttctttggtcagatgcaggacctggtgtttaataatgctctctctctaggtgagggaggcctcttgataggatgtgatctttgaagctgtatataattctcatttttaccttttaaaatgttgtacatatttgatttgaaccacggacatttgaaatgtgtaagtcaatcaagtagaaaagagctagtgaattgttcaccactttcaaggttgtgcacccacaaagcaacttgtactgtgtaatcgtccagctagagtttttacagataaagcaaatggggaagtgggtcccaacgttgctgtggtagcaggcgggtttctcttgcattggaaacagacacgtttgtaggcatttgcgtattcttgaagagactgttttatgaatcacctcttagatttatgtaatttacctaagttgttgaagtttctgtttctccttaagagaaattacaaaaattcaacattgaagcatagtttcttgttttctgttgtcaaatagtaataatgtgctgtgatgtttatgcttattcataaagatgttttactttttagtgtaatgttagttcttttaacattattttgcttaaatttgataatgcccgacaagaatatattttgctttgatttatacactgattctttgtgacaaatatgacccattaaaaatgccttttaatagactaacttaccttttgtagctaggtactcatgttcttttttaaaagatgccctttggattggattggattgatcatgtttaactcagcgtattttatggatgaaagctaaatacagatatttggcatctctaaggtggaatgagcccactccacacactgataaaattcatgcatagttttaaatgaacattaataaactcatgttgtctta

SEQ ID NO: 11 - DNA, 20 bp, synthetic construct
  source 1..20: mol_type = other DNA; note = antisense oligonucleotide
taactgacagtgagtgttgc

SEQ ID NO: 12 - DNA, 20 bp, synthetic construct
  source 1..20: mol_type = other DNA; note = antisense oligonucleotide
tacatcaggactgcctaact

SEQ ID NO: 13 - DNA, 20 bp, synthetic construct
  source 1..20: mol_type = other DNA; note = antisense oligonucleotide
atagaaacaacttacatttg

SEQ ID NO: 14 - DNA, 20 bp, synthetic construct
  source 1..20: mol_type = other DNA; note = antisense oligonucleotide
ctaaatatgtttgtttcata

SEQ ID NO: 15 - DNA, 20 bp, synthetic construct
  source 1..20: mol_type = other DNA; note = antisense oligonucleotide
ataatagtgaactaaatatg

SEQ ID NO: 16 - DNA, 20 bp, synthetic construct
  source 1..20: mol_type = other DNA; note = antisense oligonucleotide
ttaatataacccactatata

SEQ ID NO: 17 - DNA, 25 bp, synthetic construct
  source 1..25: mol_type = other DNA; note = antisense oligonucleotide
atagtgaactaaatatgtttgtttc

SEQ ID NO: 18 - DNA, 20 bp, synthetic construct
  source 1..20: mol_type = other DNA; note = antisense oligonucleotide
taactgacagtgagtgtcgc

SEQ ID NO: 19 - DNA, 20 bp, synthetic construct
  source 1..20: mol_type = other DNA; note = antisense oligonucleotide
ctaaatgggtttgtttcata

SEQ ID NO: 20 - DNA, 20 bp, synthetic construct
  source 1..20: mol_type = other DNA; note = antisense oligonucleotide
ataatagtgaactaaatggg

SEQ ID NO: 21 - DNA, 20 bp, synthetic construct
  source 1..20: mol_type = other DNA; note = antisense oligonucleotide
ttaatataatccactatata

SEQ ID NO: 22 - DNA, 25 bp, synthetic construct
  source 1..25: mol_type = other DNA; note = antisense oligonucleotide
atagtgaactaaatgggtttgtttc

SEQ ID NO: 23 - protein, 599 aa, Homo sapiens
MSGPCGEKPVLEASPTMSLWEFEDSHSRQGTPRPGQELAAEEASALELQMKVDFFRKLGYSSTEIHSVLQKLGVQADTNTVLGELVKHGTATERERQTSPDPCPQLPLVPRGGGTPKAPNLEPPLPEEEKEGSDLRPVVIDGSNVAMSHGNKEVFSCRGILLAVNWFLERGHTDITVFVPSWRKEQPRPDVPITDQHILRELEKKKILVFTPSRRVGGKRVVCYDDRFIVKLAYESDGIVVSNDTYRDLQGERQEWKRFIEERLLMYSFVNDKFMPPDDPLGRHGPSLDNFLRKKPLTLEHRKQPCPYGRKCTYGIKCRFFHPERPSCPQRSVADELRANALLSPPRAPSKDKNGRRPSPSSQSSSLLTESEQCSLDGKKLGAQASPGSRQEGLTQTYAPSGRSLAPSGGSGSSFGPTDWLPQTLDSLPYVSQDCLDSGIGSLESQMSELWGVRGGGPGEPGPPRAPYTGYSPYGSELPATAAFSAFGRAMGAGHFSVPADYPPAPPAFPPREYWSEPYPLPPPTSVLQEPPVQSPGAGRSPWGRAGSLAKEQASVYTKLCGVFPPHLVEAVMGRFPQLLDPQQLAAEILSYKSQHPSE

SEQ ID NO: 24 - protein, 596 aa, Mus musculus
MSDPCGTKPVQESNPTMSLWSLEDRHSSQGRPQPDQDPVAKEAPTSELQMKVDFFRKLGYSSSEIHSVLQKLGVQADTNTVLGELVKHGSATERECQALTAPSPQPPLVPRGGSTPKPSTLEPSLPEEDREGSDLRPVVIDGSNVAMSHGNKEVFSCRGILLAVNWFLERGHTDITVFVPSWRKEQPRPDVPITDQHILRELEKKKILVFTPSRRVGGKRVVCYDDRFIVKLAFESDGVVVSNDTYRDLQGERQEWKRFIEERLLMYSFVNDKFMPPDDPLGRHGPSLDNFLRKKPLPSEHRKQPCPYGKKCTYGIKCRFFHPERPSRPQRSVADELRANALLSPPRTPVKDKSSQRPSPASQSSSVSLEAEPGSLDGKKLGARSSPGPHREGSPQTCAPAGRSLPVSGGSFGPTEWLAHTQDSLPYTSQECLDSGIGSLESQMSELWGVRGGSPGESGPTRGPYAGYHSYGSKVPAAPSFSPFRPAMGAGHFSVPTDYVPPPPTYPSREYWSEPYPLPPPTPVLQEPQRPSPGAGGGPWGRVGDLAKERAGVYTKLCGVFPPHLVEAVMRRFPQLLDPQQLAAEILSYKSQHLSE

SEQ ID NO: 25 - RNA, 2651 nt, Homo sapiens
  source 1..2651: mol_type = mRNA
aggactcggccccatggagacgccgccggccgccgctggcgcatggcggggagctgtggcgcggggccttccaggagtctgagctatgagtggcccctgtggagagaagcctgtcctggaagccagccccaccatgagtctgtgggaatttgaggacagccacagccgtcagggcaccccaaggccgggtcaagagctggccgctgaggaggcctcggccctggaactgcagatgaaggtggacttcttccggaagctgggctattcatccacggagatccacagcgtcctgcagaagctgggcgtccaggcagacaccaacacggtgctgggtgagctggtgaaacacgggacagccaccgagcgggagcgccagacctcaccggacccctgccctcagctccctctagtcccgcggggtggtggcacccctaaggctcccaacctggagcctccactcccagaagaggaaaaggagggcagcgacctgagaccagtggtcatcgatgggagcaacgtggccatgagccatgggaacaaggaggtcttctcctgccggggcatcctgctggcagtgaactggtttctggagcggggccacacagacatcacagtgtttgtgccatcctggaggaaggagcagcctcggcccgacgtgcccatcacagaccagcacatcctgcgggaactggagaagaagaagatcctggtgttcacaccatcacgacgcgtgggtggcaagcgggtggtgtgctatgacgacagattcattgtgaagctggcctacgagtctgacgggatcgtggtttccaacgacacataccgtgacctccaaggcgagcggcaggagtggaagcgcttcatcgaggagcggctgctcatgtactccttcgtcaatgacaagtttatgccccctgatgacccactgggccggcacgggcccagcctggacaacttcctgcgtaagaagccactcactttggagcacaggaagcagccgtgtccctatggaaggaaatgcacctatgggatcaagtgccgattcttccacccagagcggccaagctgcccccagcgctctgtggcagatgagctccgtgccaatgctctcctctcaccccccagagccccaagcaaggacaaaaatggccggcggccttcaccttcatcccagtccagctctctgctaacagagagtgagcagtgcagcctggatgggaagaagctgggggcccaggcatccccagggtcccgccaagagggtctaacacagacctatgccccatcaggcaggagcctcgcacctagcgggggcagtggcagcagctttgggcccacagactggctcccacagacgctggactcactcccgtacgtctcccaggattgcctggactcgggcattggctccctggagagccagatgtcggaactttggggggttcgaggaggaggccctggtgagccgggcccaccccgagccccttacacgggctacagtccctatggatctgagctcccagccaccgcagccttctctgcctttggccgggccatgggtgctggccacttcagtgtccctgccgactacccacccgcgccccctgcctttccacctcgagagtactggtctgaaccatacccactgcccccacccacatcagtccttcaggagcccccagtgcagagcccaggggctggcaggagcccgtggggcagggcaggcagcctggccaaggagcaggccagcgtgtatactaagctgtgtggtgtgtttcccccgcacctggtggaggctgtgatggggcgcttcccacagctcctggacccccagcagctggctgccgagatcctctcctacaagtcccagcaccccagtgagtaagctgcctgtggctggcaagggcagcacccccagcctccaagggccgtcaggctgggctttgggccattgagcagcccattcccagccctgaggcccaccccagaggctggacagagggaggattcaagtcgggaaggaaacccacaaaccaaagatactgtaggattggttctggcccatgcagcacctctagctgtctgcctcagtgggtcagaagcgatcaccctgttgatacacattgtatctctgtagtttaaggagacgctgccggtaacggcgtcggtccgtggctgaggcccaaaccgtcttttctctcagagggtggggagggaggtgggggcagcagaggcctgggctgggtgccctgtgcacgccaccccacttccgccctacccctgggacgttggccttggctggctagttgggcaccgtgtgcctgccctccaagggcctcctctacgccaatgaggcctcatctgtgctctcgctgggcacgtggcttcatgtcagtaagcaagatgcttcttaataacccaccttctgccccactctattccttatcctgctgcccctgtaggggtcaagggccctccgtctacaccctcttcttctcctccatcctttattcagagtcatctcgcccttccccatgggtgggggaacctgtgtttgtttgtgtgcacatgtaaattttaaatattttaagcagaaagtccttacctcctgtaacacatcaataaagtacaatcattgtgagccctttcaa

SEQ ID NO: 26 - RNA, 2805 nt, Mus musculus
  source 1..2805: mol_type = mRNA
ttccgcgtcattgcccttaaagcacctgcccgcctgtcgcggctacgaaggtgccgtcagagcccgagactcggctccatggacaccttacagacgacgtccggcgctcagcggggagctgtgatggacacattccaagaatgtgaaatatgagtgacccttgtggaacgaagcctgtccaagaatccaaccccaccatgagtctgtggagtcttgaggacagacacagcagccagggtcgacctcagccagaccaggatcctgtggctaaagaggcccctacttccgagctgcagatgaaggtggactttttccgtaaactggggtactcgtcctctgagatccacagtgtcctgcagaagctgggagtccaagcagacaccaacacggtgctaggggaattggtgaagcatggctcagctactgaacgagaatgccaggccctgacggcccccagcccccagccccctctggtgccccggggtggaagcacccccaagccttccactctagaaccctcactcccagaggaggacagagagggcagcgacctgagacctgtggtcatcgacggaagcaatgtggccatgagccatgggaacaaggaagtcttctcttgccggggcattctgctggctgtgaactggtttctggagcgaggccacacagatattaccgtgtttgtgccatcttggaggaaggaacagcctcgaccagatgtgcctatcacagaccagcacatccttcgggaactagagaaaaagaagatcttggtgttcacgccatccaggcgggtcggcggcaagcgcgtggtgtgctatgatgaccgcttcattgtgaagctggccttcgaatccgacggagtggtggtctccaatgacacgtaccgagacctccaaggcgagaggcaggagtggaaacgcttcatcgaggagcggctgctcatgtactccttcgtcaatgacaagttcatgccccctgacgaccctttaggacggcatgggcctagcctggacaacttccttcgtaagaaaccactgccttctgagcacaggaagcagccatgcccctatgggaagaaatgtacgtatggaatcaagtgccgatttttccaccctgagcggccaagccgtccccagcgctctgtggccgatgagctccgtgccaacgctctcctctcacctcccaggactccagtcaaggacaaaagtagccagaggccttcccctgcctctcagtccagctctgtgtccctagaggctgaaccaggcagcctggatgggaaaaagctgggtgccaggtcatctccgggtccccaccgagaaggctcaccgcagacctgtgctccagctggcaggagcctccctgttagtgggggcagctttgggcccacagagtggcttgcacacacccaggactcactcccatacacctcccaggagtgccttgattcaggcattggttccctggagagccagatgtcagaattatggggcgtgcgaggaggcagccctggggagtcgggccccactcggggcccctatgcaggttatcacagctatggatccaaggtcccagcagcaccttccttttctccttttagaccagccatgggtgctggccacttcagtgtccccaccgactatgtgcccccgccacccacctacccatccagagagtactggtctgagccgtacccattacccccacccactcctgtccttcaggagccccagagacccagccccggggctggtgggggcccctggggcagggtgggtgacctggccaaagaaagggctggtgtatataccaagctgtgtggtgtcttccccccacacctggtagaagctgtaatgagacgcttcccacagctgctggatccgcagcagctggccgcagagatcctgtcttacaagtcccagcacctcagtgagtaagccagaaggtggcgcaaggggctgtcgggcatcacagatagcggtccccagcccctgcctggcctaccctggaagctggacagaaggacaagtgaagcaggcaagggaatcctcaaaccaaagataccataggattggttctggccccgcggcaccccaacccgtcccgcacaggtcagaagtgatcaccctgttgatacacattgtatctctgtcatttaaggagacgctgccggtcaggccgtccatccgtggctgatgcccaaaccctcttttttttttctcagagggccgggtgggaggcatgggggagcagaggcctgagctggaccccaccttccaccctgtccctgggacgccggcaccaccggctagttaggcaccatgtgcctgctctctgaggccccctcaagccaatgcggcctcatccctgttcacagggcatgaggcttcatgttagtaagcaagatgcttctttaagcccctcccctgcccgctctgtccacctacacaccccccccccaaccagggctccaaggccctctgtttccacacctcccatgggtgggaggacacatgtatgctgtgtacagaggcgagatttaaatattttaaatgaaaaaggttgacaaaataaaggctattgccaggcaggctggagagatggctcagtggttaagagcaccgactgctcttctgaaggtcctgagttcaaatgtcagcaaccacatggtggctcacaaacatctgtgatgagatctggtgccctcttctggggtgtctgaagacagctacagtgtacttacatacaataataaatcttttaaaaaagagagaaatttaaaagaaaaaaaaagctattgcc

SEQ ID NO: 27 - protein, 883 aa, Homo sapiens
MPGGGSQEYGVLCIQEYRKNSKVESSTRNNFMGLKDHLGHDLGHLYVESTDPQLSPAVPWSTVENPSMDTVNVGKDEKEASEENASSGDSEENTNSDHESEQLGSISVEPGLITKTHRQLCRSPCLEPHILKRNEILQDFKPEESQTTSKEAKKPPDVVREYQTKLEFALKLGYSEEQVQLVLNKLGTDALINDILGELVKLGNKSEADQTVSTINTITRETSSLESQRSESPMQEIVTDDGENLRPIVIDGSNVAMSHGNKEVFSCRGIKLAVDWFLERGHKDITVFVPAWRKEQSRPDALITDQEILRKLEKEKILVFTPSRRVQGRRVVCYDDRFIVKLAFESDGIIVSNDNYRDLANEKPEWKKFIDERLLMYSFVNDKFMPPDDPLGRHGPSLDNFLRKKPIVPEHKKQPCPYGKKCTYGHKCKYYHPERGSQPQRSVADELRAMSRNTAAKTANEGGLVKSNSVPCSTKADSTSDVKRGAPKRQSDPSIRTQVYQDLEEKLPTKNKLETRSVPSLVSIPATSTAKPQSTTSLSNGLPSGVHFPPQDQRPQGQYPSMMMATKNHGTPMPYEQYPKCDSPVDIGYYSMLNAYSNLSLSGPRSPERRFSLDTDYRISSVASDCSSEGSMSCGSSDSYVGYNDRSYVSSPDPQLEENLKCQHMHPHSRLNPQPFLQNFHDPLTRGQSYSHEEPKFHHKPPLPHLALHLPHSAVGARSSCPGDYPSPPSSAHSKAPHLGRSLVATRIDSISDSRLYDSSPSRQRKPYSRQEGLGSWERPGYGIDAYGYRQTYSLPDNSTQPCYEQFTFQSLPEQQEPAWRIPYCGMPQDPPRYQDNREKIYINLCNIFPPDLVRIVMKRNPHMTDAQQLAAAILVEKSQLGY

SEQ ID NO: 28 - protein, 903 aa, Mus musculus
MEAGPGAAEGNGPTAVILPLGPSRARGEYGVLCIQEYRKSSKVESSARNSFMGLKDHLGHDLGHLYMESTDPQMSAAVPWPMVEKPTMDTVNSGKEGKGVSEENVSSGDSEGSTSSDHESEQLSSLSVEPCSLTKTHRQLCRSPCLEPRLLKHSDILQDFKPEESQTPSKEVKKPPDVVREYQTKLEFALKLGYSEEQVQLVLNKLGTDALINDILGELVKLGNKSEADQTVSTINSVMRETSSLESQRSESPMQEVVVDDGENLRPVVIDGSNVAMSHGNKEVFSCRGIKLAVDWFLERGHKDITVFVPAWRKEQSRPDALITDQEILRKLEKEKILVFTPSRRVQGRRVVCYDDRFIVKLAFESDGIIVSNDNYRDLANEKPEWKKFIDERLLMYSFVNDKFMPPDDPLGRHGPSLDNFLRKKPIVPEHKKQPCPYGKKCTYGHKCKYYHPERGSQPQRSVADELRAMSRNTAAKTTNEGGLVKSNSVPCSTKADSTSDVKRGAPKRQSDPSIRTHVYQDIEEKLPTKNKLETRSVPSLVSIPATSTAKPQSTTPLSNGLPSGVHFPPQDQRPQGQYPPMMMATKNHGTPMPYEQYPKCDSPVDVGYYSMLNAYSNLSISGPRSPERRFSLDTDYRVNSVASDCSSEGSMSCGSSDSYVGYNDRSYVSSPDPQLEESLKCQHMHPHSRLNSQPFLQNFHDPLTRVQSYSHEEPKFHPKRPLPHLAMHLQHPAVGARSSCPGDYPSPPSSAHSKAPHLGRSLVATRIDSISDSRLYDSSPSRQRKPYSRQEGLGSWGRPSYGLEAYGYRQTYSLPDNSTPPCYESITFQSLPEQQEPTWRIPYCGMPHDPPRYQDNREKIFINLCNIFPPDLVRLVMKRNPHMTDAQQLAAAILVEKSQLGY

SEQ ID NO: 29 - RNA, 8776 nt, Homo sapiens
  source 1..8776: mol_type = mRNA
gctttctcgcggggctggctatgccgggtggcggctcccaggaatacggggtgctttgcattcaggaatacagaaaaaacagcaaagtggagtcaagtacacgtaacaacttcatgggcttgaaggatcacctagggcatgacctcggccacctttatgtggagagcactgacccacagttaagtccagctgtaccttggtcaacagtagaaaacccaagtatggataccgttaatgtggggaaggatgaaaaagaggcgtctgaagagaatgcaagctctggtgactctgaagaaaacacaaattctgatcatgagtcagaacaattgggtagcatttcagtagagccaggcttgataactaagactcacagacagctctgcaggtctccctgtttagagcctcacatactcaagcgcaatgaaattttgcaagactttaaacctgaagagtcccagactacatccaaggaagcaaagaaaccacctgatgtggtgcgagaataccaaacaaaactggagtttgcacttaagttaggttattctgaagaacaggttcagcttgtactaaacaaacttggtactgatgctttaatcaatgatattttgggagaacttgtcaaacttggaaataaaagtgaggctgatcaaacggttagtacaattaacactataacacgggaaacttcttccctggaatctcagaggtctgaatctccaatgcaagagattgtaacagatgatggtgaaaatctgagaccaatagttattgatggcagcaatgtggcaatgagccatggaaacaaagaagtattttcctgcagaggaataaaattggcagtggattggtttttggaaagaggccacaaagacattacagtttttgttcctgcttggaggaaagagcaatcccgacctgatgctctcattacagatcaggaaattttacgtaaattagagaaggagaaaatcctggtgttcacgccatcccggcgagtccaggggaggagagtggtgtgctatgacgacaggttcatcgtgaagctggcttttgagtcggacggtatcattgtgtccaatgataactacagggacttggctaatgagaagccagaatggaagaagttcatagatgaacgattattaatgtattcatttgtcaatgacaagttcatgccccctgatgaccctcttggcagacatggccccagtctggataattttctgaggaagaaacctattgttcctgaacacaaaaagcagccttgtccatatggaaagaagtgtacctatggacacaagtgcaaatattaccatcccgaaaggggcagtcagccacagcggtcagtggctgatgaactccgtgccatgtctagaaatacggcagccaaaactgcaaacgaaggaggactggtgaaaagcaacagtgttccttgtagcaccaaggctgatagcacttctgatgtcaaacgaggtgctccaaagaggcaatcagatccaagcataaggacacaagtctaccaagacctagaagaaaagcttcccaccaaaaacaaattggaaaccaggtctgtaccttccttagttagcatcccagctacttctactgcaaaaccccaaagcactacatctttaagcaatggccttccatctggagttcatttcccacctcaggatcaaagaccacagggacaatatccttcaatgatgatggcaaccaaaaatcatggaacgccaatgccttatgaacagtatccaaaatgtgactcacctgtcgacatcggatattattccatgttgaatgcatactcaaatctgagtctctcaggcccacgaagccctgaaaggcgtttctccttagacacagattatagaataagttccgtagcttctgactgcagcagtgaagggagcatgagctgtgggagcagtgactcctacgtgggttacaatgaccggtcctatgtcagctcccccgacccacagctagaggagaatttgaagtgtcaacacatgcaccctcacagccgccttaatcctcaaccgttcctgcagaatttccacgaccccttaaccagagggcaaagttacagtcacgaagaaccaaagttccatcacaagcctcctcttccgcacctggctctgcacctgccgcactccgctgtgggcgcccggtccagctgtcctggcgactacccctctcctccaagttcagcacactctaaggcaccacacctagggaggtccttggtggccacgagaatagacagcatctctgactctcgactttatgacagttctccttcacgacaaagaaagccttattcccgccaggaaggcctgggaagctgggagaggccaggctatgggatcgacgcctatgggtaccggcagacttattccttgcccgataactccacacagccgtgttatgagcagttcaccttccagagcctccctgagcaacaggagccagcctggcggatcccatactgtggaatgccgcaagatcccccgaggtatcaagacaaccgagaaaagatttatatcaatttgtgcaacatcttcccccctgaccttgtgagaattgtcatgaaaaggaatcctcacatgacagacgcccagcagctcgccgcagccattttagtggagaaatcccagctgggttattgaaagatgatgcatctttgtggtgtttagtagttttttgttcagctcaaatgctgagggaggtttgctacaatagcacatgtgatctccttctcagcaaggaggttatatagtatccatttatgtgaaatactgtatcatggaatctgtatgtatagccccacatggtggaagtatcacgggattgctttacatttaaactttttttttttaacatttcctttttaaagctatatccttggctggaaatttttccagtttgatttaatagatgtatctgtgatctttgatattaatctttggtgcatcaggggtttatatgcagcactttttatccttgttttgtgttttattaacttggtgtttgtctatcaattgcaagcaattacaataccttcagaatgtgggacatttgactagacctagcaaactgttttttcgagccaagcttagttagactcttttacagctttttaagttatttttatttggggaaagtgggcttctttgtgctataatcattatttatagaaacaaagttatactacagcactgactttatattttaaacagaatgtaagttaccagttttatgttgaaatgtgttacagtatatatatattagaatgatttacaatatggcacttttcgatgtgttatttttgtttggatttttttttctgttaagaaattagttaatttaatatggtcaatttaaaagaaagcagatgcaatcaatggaaaaatgtttccattttttaaaaatgaataaggcaaaagctgtaactgttacaggttagagctttgttatccagctatgatgtgcttcttgacagtagaagtggaattgaattcctagatttccattaacctgtatttttaatatgtctgtctttttgttttggggcacaacaatactggataaaataaccctttcacagcacttgcctgtttttaatgaatctaattattcacaatgcaacttttatatttaacatactctttagctttcctgctatttatcaaggctggcctgaggtgggtttatgtgttgaggttatgcaacatttcttgatactgcactatagagaaatggtgatggaggagttgtaaatggtaacttaaaatttttgtaagatattgtatattttccattttcctgaaggtagttttcttgggggggcctgttatattattaaggccagactcttgccacaaatagtgtagttttagatacagactaaggtctgttctagtattagtaagggatatttctggtttcaaagtcatgggttttgctagtggtgaatacatttctgcggagtagaagatagattttgcagtcagtggcagacagttgtgtgattgacatcacttgactgttgcgtccaggttttgaattgtacttcacgtaacagatgcattcagatctttttctgtagtctgcttagatgccctggctattctgattatcctacatgctacagtttgaagtgaagccctgaaaaaccagaaagtaccttttactgttgatacaaattgtatctttttaactataagaactattttgatttgtagatctagttaaaacacaagtatgtaactatgattagacttttgggcaacattttatcccttatttaaatacaaatttttaaagtaaaattgaggtctagaatagattagaaaataaaaataacaatttagataaatagaaatgtctgtcttagttttatataatatattaaaacacagtaaataaatttattggcattttctttctcctaaaacttacctagtgtgaacttaaaataaaggtaaaatgctgcctgaaaataatgtccaagcacctttgactaggataacattttcactacttgtgtgacactgtgtgttgcacgaagtaggatttgggtatacagtaaatgcttctaaaaggcattgtgcatattgacataaccaataatctgaaccgtgttcagcaaacttaattcaggaaagtggtattctacacaattattgctgttgtgtttgaaatgagtgtggcactcatctgtatccagaaataatatgggtgaggccacacaacccattctgagtggtgtctgtctgaaagcaaccctactcgcatgtgaaattgttctccttgatttggtcactataaagcaagtttaaatgtagaggctaactcagtgccaaaaacagggttacaaatgtgtagtatcttttattttagtcatattctaagacttctttttagtatgaaatcacttttaaattatacatgtaggttttgcttccattttcttcattttaccattttaattatttgaacattcgccaaattttacatttatttaaatgagatcttaggtgagatgtgtgtgacactttgaatttgaccttcttgtgttattagctgactatttgtcattgcctcatggattttaaattatgggaaaatagtgtagccagctgccacctctactgaagtgagtagctctgaactacccacactaaatccttcagtgtaattaattatgagtttaaaaatagcagttttcttatgtgaagaggacagtttgtcccctttttttgaagcaccgatgttgcgttcagagctgtagaatgagataattggcagactttaggtacagcaaattcttacttatctaaagcaataagtcaaaggagtccatcattaaattaaatccatagctgatcacaagccttcattttagccaaaactttctctctaaccaaatcttttaccagacttgctaataaataaccagagagatgtgttaataagtgaagttgccagaaatggtcaactgatcggaaaaaaaaggattcagactggagtattttgcccctgaataattgacagttgactgtgctttacacagtaactagccagtctgttgtctctgtgtcttagtccagagggaatagtacccaattggccaaatactggcccttagtatctcctcctttcttgcatgggatacagacgttttcagtcttgtttttatgatctctctctatatcctgataagagtttgtcattgacttacacatttggaagaaatgcacaccagtgtaatatatttgatactggtggaaacttgaactttgtgtttttatgaaaattcatttatgagaatatgtaatataactgaagagtattttatgtatatctatatacacaaatatgtatttgttatgaggtattaaaaacaggggttggggggagtgcttctgatggctaacttttctctaattaaactatgtttctttgagttgtgaacgaccgagtctggggtctggacggccaatgataagatttagaaccacttggatggaaagcagttcttcactggttttattcttggtattttcaaagaattattttgatatttttaatagaatgtgtaattttaaaatacacaaaaaacttaaagtagtattgattatacaaataattatttaacatgtcttatggatgtatctatatgtatatagacagtaatatatttataaaacaaatatactttgcttatgttatagctcttagtttgtgacaggtgggaggatggctctgggtgtgtgtgtgtgtgtgtgtgtgtgtgtgtgtgtgtgtgtgttttgaaaactctcaagctgttttccctctgatttacaatggtatttactttaaagtatgtttggttttcattattctttttgctctccaacttccttattcaagataaaataagacatacagttttctggccattctgttggtgtgtggtgcacccattttattgtcatctaactcctggagaattcccacgtgacctgaaatcaaacagattctggctggacatatgcttatgttccaaatatattaaagatgttaattcagctaacagttaagtttccaaggtatacaccaacaaataaaatgaggtattaaaaagagatggattacacacatgcattagaataagagaaaacagtagtgttaataaaagtaaagaaacatacactatcttagccccctagggcaggggttgactttttctgtaaaggatcagatagtaaataatacaggaatcatatggacttcaaatgccattgtaaaaactactcagctctgcctttagagcataagaacagccacagataacatgtaaattagtgtggctgtgttccaataaaactttatttacagaaacgggaagccggtcagattgggcctgtgggccataatttgctgatctcaagcagtaaatcctggtatatgttaatagaagaaatcataattgcatttcagttgacattaaaagaaaatctggtagtttttgatgtccttcaaaagaggattgttagacattgatgttaaagcatcttaattcatttgagttttcttacctgtttacacccattatttattagagatatttcttgtgtttaaccacaaaaaaaagcactctgttaaaatgttttaatatgtattgaatttctttcataaacttttcatttctgttgataaatgggaatcccttaccaaccttttgttttttaaaagtctcatagaccaaaaaaaatctgttgcagcatttaattagccacagatacattttggctgcatttaccagttacatttttccattggttttggcttctaataaataacatatctgccattctttaaaaatgattttaaagaagataaatatattgtaatttcacatgctatagctttattctgtaagattaaaaattgtgactagtataattgtagctataatgtgagtggcatgttacaatgtaactctttatgagaaataaaatgtatctctgctttgtctgtccagatctttaggatttttagatgccttgggactgtccttggtgaatgatattcttcatatgatcatatgtaattttgaattcgttggaagtacacgctgctgagcatgtttattcacagtgctttataccgggtgttgcatcagtaatcattttcataagaacatttaaacagcatgaacatcatcatccacttaaatagttaaactttcttttaaaattggaatgcaactgtaggttttaacaatgtttattgttttttaagtggttactttgtttttccttaatactttctgttaacttaattattactcctgttgcagtgttactgttatgtattagaagtggcttttccccctaagatccttagtcttttaaagacaatttaaggtattggccatttggcagtagaaaatgtgcatgttttaacttggttttataaaatctgtaatgtttcacttcttgaaccatgtaccaaatttgccaattttctgtccaagtgtttcagatgaataacaaaacgctgttcattgaagctttcgccacctttcttaaagcagcgtatgttccaagggaaaaaggcattgaaaagcaatcgtttgtttttatgaagaataggtgttcagattccttcagtttttttgaaattagaaatttcttaccttatgtgaaatattcacaaacgtgcacacttctgcagagacaaagcatttcactgcacgtgtaccaggttattgattttatcttttcctttcagggttttgtcctcccaaaccagagtcatatgctgctagtagaattttttatttgatcctgcgaacttttcttataggaaaagtaaggcaaaggatgtgtagtgcaaccatctgataaactagtgtgattgtatttatcctctgttctgtgtatttctgtaatggaatctttacaattcccaaaacggtattttagacctactggaaatctgtatcgaaacagctatgtgattctgccactgagaaaaaaaaaatttttaattcgtttttcttatgctggtttgtttttctttaatgaagaaattgatctcatatggcatcatagatgctaaataaataaaagcatcatacttctctagtttgcctgcattcagtggctaacattatgagcattgtgtaagataaacacatggtcagtatcaatgtaaatgttagagccatgattaattcctatgaaaattgaaattaaatgtcaaagacaactagacataa

SEQ ID NO: 30 - RNA, 8844 nt, Mus musculus
  source 1..8844: mol_type = mRNA
aggcgcgggaggcccgcggggcaggggaggccgcgcccgagagcggagctcaggatccgccggagccggagccagagcggccacgctcagggaactccaggcccaggcggctccgacccccgaggtcgagtggcgcagcgcccgccgccccgaacactgagcgggaaagccgagcgcatcctgcccgcgggcggcgccagcccccgtggggaattcgacgaggggaggccgggcccggaggcctagaacgccggtccagtagctccagcccgcccgagggccagggccagcgaacatggaggcgggcccgggcgccgccgagggaaacggacccacggctgtgatcctgccgctcggaccctcgcgcgctcgtggggaatacggggtgctttgcattcaagaatacaggaaaagcagcaaagtggagtcaagtgcacggaacagcttcatgggcctgaaggatcacctggggcatgatcttggccatctttatatggagagcactgacccacagatgagtgcagctgtgccttggcctatggtagagaaaccaacaatggatacagtcaattcggggaaggaaggaaaaggggtgtcagaagagaatgtgagctccggcgactctgagggaagcacgagttctgatcatgagtcagaacaactgagtagcctttcggtagagccatgctcattaaccaagactcacagacagctatgtcgctctccctgcttagagcctcgcctactgaaacacagtgacattttgcaagactttaaaccagaagagtcccagactccatctaaggaagtgaagaaaccccctgatgtggttcgagaataccaaacaaaactggagtttgcacttaagttaggttattctgaagaacaggtccagcttgtgctaaacaaacttggtactgatgctttaatcaatgatatattgggagaacttgtcaaacttggaaataaaagtgaagccgatcaaacagttagtactattaacagcgtaatgcgagaaacctcatccctggagtctcagaggtctgaatctccaatgcaagaggttgtagtagatgacggtgagaatctgagaccagtagttattgatggcagcaatgtggcaatgagccatggaaacaaagaagtattctcgtgccgaggaataaaattggcggtggattggtttttggaaagaggccataaagatatcacggtctttgttcctgcttggagaaaagaacagtcccgccctgacgccctcatcacagatcaggaaattttacgtaaactagagaaggaaaaaatcctggtattcacaccatcacggcgtgtccagggcaggcgagtggtgtgctatgatgacagattcatcgtgaagctggcttttgagtccgatggtataattgtgtccaatgataactacagagatttggcaaatgagaaaccagaatggaagaagttcatagatgagcggttattgatgtattcctttgtcaatgacaagttcatgcccccagatgaccctcttggcagacatggcccaagtctggataattttctgaggaagaaacccattgttcctgagcacaaaaagcagccttgtccctatggaaagaagtgtacgtatggacacaagtgcaaatactaccacccagaaaggggcagtcagcctcagcggtcagtggctgatgaacttcgtgccatgtctagaaacacagcagccaaaactacaaatgaagggggactggtgaaaagcaacagtgttccttgcagcaccaaggcagacagcacttcggatgttaaacgcggtgctccaaagaggcagtcagacccaagcataaggactcacgtctaccaagacatagaggagaagcttcccaccaaaaacaagttggaaaccaggtctgtaccttccttagttagtatcccggccacttctactgcaaaaccccaaagcactacacctttaagcaatggccttccatctggagttcatttcccacctcaggatcaaagaccacagggacaataccctccaatgatgatggcaaccaaaaatcatggaacgccaatgccttatgaacagtatccaaaatgtgactcccctgttgacgttggatattattccatgttgaatgcatattctaatctgagtatctcaggcccccgaagtcctgaaaggcgtttctcactagacactgattacagagtaaactctgtggcttcagactgcagcagtgaagggagcatgagttgtgggagcagcgactcctacgtggggtacaatgaccgctcctatgtcagctctcctgacccacagctggaagagagtctcaagtgtcagcacatgcacccccacagccgccttaattcccagcccttcctgcagaatttccacgatcccttaaccagagtccagagttacagtcacgaagaaccaaagttccatcccaagcgtcctcttccacacttggctatgcatctgcagcaccctgccgtgggtgcccgctccagctgtcctggcgattacccctccccaccaagttcagcacattcgaaggcaccacacctagggaggtccttagtggccacgagaatagacagcatttctgattcccgactctatgatagttctccttcaagacaaagaaagccttattctcgccaggaaggcctaggaagctggggtaggccaagctatgggctggaagcatatggctatcggcagacgtactccttacccgataattccacgcccccatgctatgagtcgatcaccttccagagcctgcctgagcagcaggaacccacctggagaatcccctactgtggaatgccacacgatcctccaaggtaccaggacaaccgagagaagatttttatcaatttgtgtaacatcttcccccctgaccttgtgaggctcgtcatgaaaaggaatcctcatatgacggatgcccagcagctcgccgcagccatcttagtggagaaatcgcagctgggttactgaaagcatgatgcatctttgtggtgttgagtagttttttgttcagctcagttgctgagggaggtttgctacaatagcacatgtgatctccttctcggcagggaggttatatagtatccatttatgtgaaatactgtatcatggaattgtatggaaccccacttggtggacttatcacgggattgctttacattcaaactttttttttttttttttaacatttcctttttaaagctatatacacttggctggaaatttctccagtttgatttactagatgtatctgtgatctttgatattcctctttggtgcatcaggggtttatatgcagcactttttatccttgtttcctgtcttattaacttggtgtttgtctgtcaactgcaagcaattgcagcaccttcagaatgtggaggtaccgggctagacctagcaaacaatgtcctcaagccaagcgtagctagaatcctttacagctttttaagttatttttatttggggaaagtgggcttctttgtgctataatcattatttataggaacaaagatatactacagcactgactttatatttttaaaaaatttaagcttccagttatgttaaaatggaaatagtacatattagagtgattcccggtatggcactttttattattttatttttgtttggatgtttcctgttaagaaaattagttattttaaatggtcagtttaaaagaaagcagatgcaatcaatcgaaaaaaaatgtttcttttttatgaataaggcaaaagctgtgactattacaggttagggctttgctttctagctaaaatgtgctttttgacagtagaagtgggattgaagtccttgatttccattaacatgtatttttaatctgtctttttgtgggaggcacagtactggatgaatagccctttctcagtacttgcctgtttttaatgaatccaagtattctcaatgcaacttttatattgaatacactctagcttcctgctatttactgaggctggcctgaggtggtctgatgtgttgaggatatgcaacatttactgatactgcactagagaaatggcaatggaggacttgtaaatggtaacttaaagtttttgtaagatattgtatattttccattttcctgaaggtagtttttttggggagcctgctataatattaaggccagactcttgccacaaatagtgtagttttagatacagactaaagtctgttctagtattagtaagggatatttctggttgcaacgtcatggcttttgcttgctgtagcgacctttctgagcatcagagatggatctatggcagacagtgcagacagtgctgtgatggacagaggctgcctctgacgttacttgttgcagcgacaagtctagctctgctcctgtagtcagcctggaggcttggtctagatgctcctgcagtctgagagaggcaaagccctggaaaccagaaagtaccttttactgttgatacaaattgtatctttttaacaataagaactattttgatttgtagatctagttaaaaacacaaatgtgtaactataattagacttttgggcaacattttatcccttatttaaataaaaaaaatttttaaaggaaaattgaagtctagaataggatagaaaataaaagtaacaattaaggtaaataaaggtgtctgtcttagttttatatattaaaatatattaaataaatttattggcattttctttttcctaaaacttacctagtgtgaacttaacttaaaataaaggtaaaatgctgcctgaaaataatgtccaagcatcttcgactaggataacattttcactacttgtgtgacactgtgtgttgcatggagtaggatttgggtacacagtaaatgcttctaaacggcattgtgcatattagcatatccaataatctgaaccatgttcagcaaacttaattcaggaaagtgatgttctacagttactgctgttgtgtttgagtgagcgtggcacacatctgttcccggagtgctgcaggtggtgccaccccagccctcccgagtgctgtgtctgagagtgacacagccgacctgtgaaactgtccttgattctctcagtcataatctaaaggacaagttgaaatgtggaggctaagtgaatgccaagaacagggttgcaaatgtggggttcctcatacccaggctgcccagccacattgtgaggccaggctaggaagtcagttaatgaacatgtcacttttgcttcatattagcactgtgattgtttggaaatgggcacacttgactaaaatggtttaagcgagaccttaggtaaaaaggatatgacttaaaatttggccttcttacatttttagctgaagttgccctctttttcatctctgccagtgtgtgtcatggagtgggtagctctgacccacccactcctacatttctcagtgccattggctgtgtgctaagaaaaggttttcttatgacaagaggacagtctgtctgtcccctttgataaagcaccaatgctgctttcagacgttaagaataaggtgattggcaaattttagctacatcagtttctcaaaaaacaaaacaaaacaaaaacctcaggtaataagtaaaaggagtccattatcaaatttgtagctgatcataaaccttaattttagctagaatatttcttcccaatctctaatttctatttaagagactagctaaaataaataaataacctgaaatggtgtgctaatgaatagtaaaagtcagaattggtcagctgattaaaaaggactcagactggaatattctgcccctgaataatagacagtcaactgtactttatgcagtaatagcagtttgttgtccctgtgtcttagtccagagggaatagtacctaactggccaaaatggccctcagaatttcctcttttcttgcatgtaatatagacatttcttgttatcctaatgggagtttgtcactgacctaaacagtgaaagtaatggtcgccagtaaaatatttgacactggtgacaacttgaatttttgatttcatgaaaatacatttatgaaaatatgtaattacctaaagagggtgttttatatatacacgtttgttatgaagtattaaaaaatagggggttgtctttcaatggataacattttcctgattgaacggtgtctttgagttgtgaatgaccaagtctagggtctatttgaccaatgataagattcagaacctcttacatggaaagaaacacttggttttattcttggtatttttaaagattattttgataattttaatagaatgtgtaatttttaaatacacaaaagtagtattgattatacaaatgattatttaacatgtcttttatggatgtatctatatgtatatagacagtaatatatttataaaacaatatactttatgttgtattttttagtttgtaatgaatgtaagtatgactgtgtgtatgtgagcaagcactcacatgtgtgtacatgtgcacacacgtgttgatgtgtctgtctgcctgtgtttgaatgctgaaacctctttccctgacttgctgggatttactctaaaatgtatttgggttttgctccttttaatacccttattccttattcaagataaaataagaggtacagttttcttgtctgtctgttgccagatggctcttccattgtattaatctctaattcttagagaaggcctgacatcaagcagattatgactggagataatgactatgttccaaatatattaaaagtgaaccccgctgtgatgtgaaaatttcaggatccacaccaatgaacagaataagcctagaagatcgagtcatccacacaccagagttcgaggaggcctgggacctgtgacaaggaagacacgtgtgttctagatgctctctctataggatctggtagtcaataattcaggcttctctgagaatcagatagtctctttactgtacacctttgcctttacagtgtgacagccacaggtagcatagagatgaaaatgtgaccttttaaataaaattttatttacagaaacaagcaacaggccagtttttacctgtgggccattccccagccctgtccttgagggaaaaaaagccagacatcttaagctgtaaattcttgtgcatgttaatataatcaacaatagctgtatctcagcagccatctagaggcagtatgacgagtcactggtgtccttcagaagatggctgtgcaacagtcacagggaagcatttgttacgttcagcacatccatcatttgagatgtcacttatctagccaccaagaaatctataaaagaaaggtatcaggactgggaattttgcttaagttcttatttttaagtaggactcctttatcttttgtttctcagtggcctcgtgggccaaaaaccagcctttttttttttttaactcagccacatgtttttcaagattgcatttgtcagttacgtttttctgttaggtttttgtcttctgatgcttaacagacttacccttctttacaagtgagtttaaagattaacatactataacttcacagtgtcagatttctctgtgatgtttaaagctgactagaccaatgagtgtattttttacattgtcactcttaataagaaacatgcgtcttctttctctgtctgaatgttcactatggagtgtttagctaccttagggcctgccatgggagtgatgctctcatgagcacctgcgagtctgaattgattgaaggtacacaccactgaacatgctcattcacactgctccattcatggtatctcagcaataacactatctttacaggattgttaaatagctacgaaaactaccgcctacttaagtagttacaccttcttttaaaattggagtgcagtcctggctttatcagtattgatgttttgtctgttacaccctctcacctcctgcctgtcacccatgttatgtcaacactgtcatatttatacatggcttttcccctaggatcctcaatccttcagacctaaacacaatttcaggttttgaccatttgacagtagaaaatgtctatgcatgttttcaatccttacaaacctgtgaagttttatttcttaatccatgtactgaactttctgtccaggtgaacaagatgcttcccagaaaagcttttcccacttctatctaaagcagctcatgtctttaagacaaagaagtgcgcggttgttttgtaaggtataaacacatacatgggtgtatgtatgtatgtatgtatgtatatatttcctctggggtttttttaattataaattttcaaccttctgtgaaatactcacaaatggtcaaatactgcagacagggtataccctcgctgtcaggtcttctattcctcccaactgtagctttttgccagtagagaatttccttactcatccttcaagcttttcttacaggaaaaataaagtaatgaatatgtttagatcaaccattttataaacatattattctgtttatcactatctgttctgtatgtttctgtatagaacttttacaattcccaaaacagtggaaatagctatatgattctgccatagagggggagattctaagatatccatctttcttgtggcaggtggttgttacatgaaaaaatagatctcatatgatggcatagattctaaataaacaaagcatttccttttctgttcccctggctttctcagattctgtgattagtgacattgggctacacatgttcagcattgatgtaaatgttagagccacaattaattcctattaaactgaaattaaatgtcaaaaattagtcatgactcaaaa

SEQ ID NO: 31 - DNA, 20 bp, synthetic construct
  source 1..20: mol_type = other DNA; note = antisense oligonucleotide
aatacagggcaaatggtcta

SEQ ID NO: 32 - RNA, 125 nt, Homo sapiens
  source 1..125: mol_type = mRNA
acactcactgtcagttaggcagtcctgatgtatctgtacatagaccatttgccttatattggcaaatgtaagttgtttctatgaaacaaacatatttagttcactattatatagtgggttatatt

SEQ ID NO: 33 - RNA, 125 nt, Mus musculus
  source 1..125: mol_type = mRNA
acactcactgtcagttaggcagtcctgatgtatctgtacatagaccatttgccctgtattggcaaatgtaagttgtttctatgaaacaaacccatttagttcactattatatagtggattatatt

SEQ ID NO: 34 - RNA, 125 nt, Bos taurus
  source 1..125: mol_type = mRNA
atactcactgtcagttaggcagtcctattgtatctgtacatagaccatttgctttgtattggcaaatgtaagttgtttctatgaaacaaacatttttagttcactattatatagtgggttacgtt

SEQ ID NO: 35 - RNA, 125 nt, Gallus gallus
  source 1..125: mol_type = mRNA
acactcactgtcagtcaggcagtcctaatgtatctgtaaatagaccatttgcctggtgttggcaaatgttagttgtttctatgaaacaaaagtattttgttcactatcatatagtgggttatgta

SEQ ID NO: 36 - RNA, 125 nt, Mauremys reevesii
  source 1..125: mol_type = mRNA
acactcactgtcagttaggcagtcctaatgtatctgtaaatagaccatttgccctgtgaaggcaaatgtgagttgtttctatgaaacaaaagtatttagttcactatcatatagtgggttatgtt

SEQ ID NO: 37 - RNA, 48 nt, Mus musculus
  source 1..48: mol_type = mRNA
agttgtttctatgaaacaaacccatttagttcactattatatagtgga

SEQ ID NO: 38 - DNA, 19 bp, synthetic construct
  source 1..19: mol_type = other DNA; note = antisense oligonucleotide
aactaaatatgtttgtttc

SEQ ID NO: 39 - DNA, 18 bp, synthetic construct
  source 1..18: mol_type = other DNA; note = antisense oligonucleotide
atagtgaactaaatatgt

SEQ ID NO: 40 - DNA, 19 bp, synthetic construct
  source 1..19: mol_type = other DNA; note = antisense oligonucleotide
aactaaatgggtttgtttc

SEQ ID NO: 41 - DNA, 18 bp, synthetic construct
  source 1..18: mol_type = other DNA; note = antisense oligonucleotide
atagtgaactaaatgggt